European Patent Application EP 4 227 403 A1, published August 16, 2023. Title: EXOSOME AND PREPARATION PROCESS AND USE THEREOF. Applicant: Ascension Medical Biotechnology Co.,Ltd. The sequence listing filed with the application follows.

SEQUENCE LISTING (14 sequences)

SEQ ID NO: 1 - DNA, 16 bp, synthetic construct
  misc_feature 1..16: note = Forward primer COL1A1-F of COL1A1 gene for quantitative real-timePCR
  source 1..16: mol_type = other DNA
gtcagatgggcccccg

SEQ ID NO: 2 - DNA, 20 bp, synthetic construct
  misc_feature 1..20: note = Reverse primer COL1A1-R of COL1A1 gene for quantitative real-timePCR
  source 1..20: mol_type = other DNA
caccatcatttccacgagca

SEQ ID NO: 3 - DNA, 21 bp, synthetic construct
  misc_feature 1..21: note = Forward primer COL3A1-F of COL3A1 gene for quantitative real-timePCR
  source 1..21: mol_type = other DNA
gaggatggttgcacgaaacac

SEQ ID NO: 4 - DNA, 21 bp, synthetic construct
  misc_feature 1..21: note = Reverse primer COL3A1-R of COL3A1 gene for quantitative real-timePCR
  source 1..21: mol_type = other DNA
cagccttgcgtgttcgatatt

SEQ ID NO: 5 - DNA, 18 bp, synthetic construct
  misc_feature 1..18: note = Forward primer ELN-F of ELN gene for quantitative real-time PCR
  source 1..18: mol_type = other DNA
caggtgcggtggttcctc

SEQ ID NO: 6 - DNA, 20 bp, synthetic construct
  misc_feature 1..20: note = Reverse primer ELN-R of ELN gene for quantitative real-time PCR
  source 1..20: mol_type = other DNA
ctgggtatacacctggcagc

SEQ ID NO: 7 - DNA, 20 bp, synthetic construct
  misc_feature 1..20: note = Forward primer 18s-F of 18s rRNA gene for quantitative real-time PCR
  source 1..20: mol_type = other DNA
gtaacccgttgaaccccatt

SEQ ID NO: 8 - DNA, 20 bp, synthetic construct
  misc_feature 1..20: note = Reverse primer 18s-R of 18s rRNA gene for quantitative real-time PCR
  source 1..20: mol_type = other DNA
ccatccaatcggtagtagcg

SEQ ID NO: 9 - DNA, 20 bp, synthetic construct
  misc_feature 1..20: note = Forward primer IL-6-F of IL-6 gene for quantitative real-time PCR
  source 1..20: mol_type = other DNA
acccccaggagaagattcca

SEQ ID NO: 10 - DNA, 20 bp, synthetic construct
  misc_feature 1..20: note = Reverse primer IL-6-R of IL-6 gene for quantitative real-time PCR
  source 1..20: mol_type = other DNA
gatgccgtcgaggatgtacc

SEQ ID NO: 11 - DNA, 20 bp, synthetic construct
  misc_feature 1..20: note = Forward primer IL-1beta-F of IL-1beta gene for quantitative real-timePCR
  source 1..20: mol_type = other DNA
gcagccatggcagaagtacc

SEQ ID NO: 12 - DNA, 24 bp, synthetic construct
  misc_feature 1..24: note = Reverse primer IL-1beta-R of IL-1beta gene for quantitative real-timePCR
  source 1..24: mol_type = other DNA
agtcatcctcattgccactgtaat

SEQ ID NO: 13 - DNA, 22 bp, synthetic construct
  misc_feature 1..22: note = Forward primer TNF-alpha-F of TNF-alpha gene for quantitative real-timePCR
  source 1..22: mol_type = other DNA
tagcccatgttgtagcaaaccc

SEQ ID NO: 14 - DNA, 21 bp, synthetic construct
  misc_feature 1..21: note = Reverse primer TNF-alpha-R of TNF-alpha gene for quantitative real-timePCR
  source 1..21: mol_type = other DNA
ttatctctcagctccacgcca